European Patent Application EP 4 644 544 A2, published November 5, 2025. Title: Generating recombinant immunoglobulins using an expression library. Applicant: NANTBIO, INC. Application EP. The sequence listing filed with the application follows.

SEQUENCE LISTING (120 sequences)

SEQ ID NO: 1 - DNA, 58 bp, synthetic construct
  misc_feature 1..58: note = Artificial Sequence for VH CDR1
  source 1..58: mol_type = other DNA
ggcttaggtctcatttcrvtagttacgctatgcattgggcgagacgaggtctgaacgg

SEQ ID NO: 2 - DNA, 58 bp, synthetic construct
  misc_feature 1..58: note = Artificial Sequence for VH CDR1
  source 1..58: mol_type = other DNA
ggcttaggtctcatttctctrvktacgctatgcattgggcgagacgaggtctgaacgg

SEQ ID NO: 3 - DNA, 58 bp, synthetic construct
  misc_feature 1..58: note = Artificial Sequence for VH CDR1
  source 1..58: mol_type = other DNA
ggcttaggtctcatttctctagttackkgatgcattgggcgagacgaggtctgaacgg

SEQ ID NO: 4 - DNA, 58 bp, synthetic construct
  misc_feature 1..58: note = Artificial Sequence for VH CDR1
  source 1..58: mol_type = other DNA
ggcttaggtctcatttctctagttacwmtatgcattgggcgagacgaggtctgaacgg

SEQ ID NO: 5 - DNA, 58 bp, synthetic construct
  misc_feature 1..58: note = Artificial Sequence for VH CDR1
  source 1..58: mol_type = other DNA
ggcttaggtctcatttctctagttacgctatgavttgggcgagacgaggtctgaacgg

SEQ ID NO: 6 - DNA, 54 bp, synthetic construct
  misc_feature 1..54: note = Artificial Sequence for VH CDR2-n
  source 1..54: mol_type = other DNA
ggcttaggtctcgttcathcattagtggtagtggacgagacgaggtctgaacgg

SEQ ID NO: 7 - DNA, 54 bp, synthetic construct
  misc_feature 1..54: note = Artificial Sequence for VH CDR2-n
  source 1..54: mol_type = other DNA
ggcttaggtctcgttcavktattagtggtagtggacgagacgaggtctgaacgg

SEQ ID NO: 8 - DNA, 54 bp, synthetic construct
  misc_feature 1..54: note = Artificial Sequence for VH CDR2-n
  source 1..54: mol_type = other DNA
ggcttaggtctcgttcagctattyggggtagtggacgagacgaggtctgaacgg

SEQ ID NO: 9 - DNA, 54 bp, synthetic construct
  misc_feature 1..54: note = Artificial Sequence for VH CDR2-n
  source 1..54: mol_type = other DNA
ggcttaggtctcgttcagctattdatggtaatggacgagacgaggtctgaacgg

SEQ ID NO: 10 - DNA, 54 bp, synthetic construct
  misc_feature 1..54: note = Artificial Sequence for VH CDR2-n
  source 1..54: mol_type = other DNA
ggcttaggtctcgttcagctattagtwmtagtggacgagacgaggtctgaacgg

SEQ ID NO: 11 - DNA, 54 bp, synthetic construct
  misc_feature 1..54: note = Artificial Sequence for VH CDR2-n
  source 1..54: mol_type = other DNA
ggcttaggtctcgttcagctattagtkggagtggacgagacgaggtctgaacgg

SEQ ID NO: 12 - DNA, 54 bp, synthetic construct
  misc_feature 1..54: note = Artificial Sequence for VH CDR2-n
  source 1..54: mol_type = other DNA
ggcttaggtctcgttcagctattagtggtrrtggacgagacgaggtctgaacgg

SEQ ID NO: 13 - DNA, 52 bp, synthetic construct
  misc_feature 1..52: note = Artificial Sequence for VH CDR2-c
  source 1..52: mol_type = other DNA
ggcttaggtctcgtggarvkagtacttactacgcgagacgaggtctgaacgg

SEQ ID NO: 14 - DNA, 52 bp, synthetic construct
  misc_feature 1..52: note = Artificial Sequence for VH CDR2-c
  source 1..52: mol_type = other DNA
ggcttaggtctcgtggaggtnatacttactacgcgagacgaggtctgaacgg

SEQ ID NO: 15 - DNA, 52 bp, synthetic construct
  misc_feature 1..52: note = Artificial Sequence for VH CDR2-c
  source 1..52: mol_type = other DNA
ggcttaggtctcgtggaggtrvaacttactacgcgagacgaggtctgaacgg

SEQ ID NO: 16 - DNA, 52 bp, synthetic construct
  misc_feature 1..52: note = Artificial Sequence for VH CDR2-c
  source 1..52: mol_type = other DNA
ggcttaggtctcgtggaggtagtactvrttacgcgagacgaggtctgaacgg

SEQ ID NO: 17 - DNA, 53 bp, synthetic construct
  misc_feature 1..53: note = Artificial Sequence for VH CDR3
  source 1..53: mol_type = other DNA
ggcttaggtctctccgtgrtckcnnkngstttcgcgagacgaggtctgaacgg

SEQ ID NO: 18 - DNA, 58 bp, synthetic construct
  misc_feature 1..58: note = Artificial Sequence for VL CDR3
  source 1..58: mol_type = other DNA
ggcttaggtctctgcagdsgdmtrvtdsgccttwcacttcgagacgaggtctgaacgg

SEQ ID NO: 19 - DNA, 58 bp, synthetic construct
  misc_feature 1..58: note = Artificial Sequence for VL CDR3
  source 1..58: mol_type = other DNA
ggcttaggtctctgcagbwtdmtrvtdsgccttwcacttcgagacgaggtctgaacgg

SEQ ID NO: 20 - DNA, 58 bp, synthetic construct
  misc_feature 1..58: note = Artificial Sequence for VL CDR3
  source 1..58: mol_type = other DNA
ggcttaggtctctgcagdsgdmtrvtnwtccttwcacttcgagacgaggtctgaacgg

SEQ ID NO: 21 - DNA, 58 bp, synthetic construct
  misc_feature 1..58: note = Artificial Sequence for VL CDR3
  source 1..58: mol_type = other DNA
ggcttaggtctctgcagbwtdmtrvtnwtccttwcacttcgagacgaggtctgaacgg

SEQ ID NO: 22 - DNA, 58 bp, synthetic construct
  misc_feature 1..58: note = Artificial Sequence for VL CDR3
  source 1..58: mol_type = other DNA
ggcttaggtctctgcagdsgdmtrvtdsgcctykgacttcgagacgaggtctgaacgg

SEQ ID NO: 23 - DNA, 58 bp, synthetic construct
  misc_feature 1..58: note = Artificial Sequence for VL CDR3
  source 1..58: mol_type = other DNA
ggcttaggtctctgcagbwtdmtrvtdsgcctykgacttcgagacgaggtctgaacgg

SEQ ID NO: 24 - DNA, 58 bp, synthetic construct
  misc_feature 1..58: note = Artificial Sequence for VL CDR3
  source 1..58: mol_type = other DNA
ggcttaggtctctgcagdsgdmtrvtnwtcctykgacttcgagacgaggtctgaacgg

SEQ ID NO: 25 - DNA, 58 bp, synthetic construct
  misc_feature 1..58: note = Artificial Sequence for VL CDR3
  source 1..58: mol_type = other DNA
ggcttaggtctctgcagbwtdmtrvtnwtcctykgacttcgagacgaggtctgaacgg

SEQ ID NO: 26 - protein, 6 aa, synthetic construct
  REGION 1..6: note = Clone 801 CDRH1
NSYAMH

SEQ ID NO: 27 - protein, 10 aa, synthetic construct
  REGION 1..10: note = Clone 801 CDRH2
AISGNGGSTR

SEQ ID NO: 28 - protein, 8 aa, synthetic construct
  REGION 1..8: note = Clone 801 CDRH3
DRFRKVHG

SEQ ID NO: 29 - protein, 6 aa, synthetic construct
  REGION 1..6: note = Clone 801 CDRL3
DATFPL

SEQ ID NO: 30 - protein, 6 aa, synthetic construct
  REGION 1..6: note = Clone 802 CDRH1
GSYAMH

SEQ ID NO: 31 - protein, 10 aa, synthetic construct
  REGION 1..10: note = Clone 802 CDRH2
AISGSGGSTR

SEQ ID NO: 32 - protein, 8 aa, synthetic construct
  REGION 1..8: note = Clone 802 CDRH3
DLYRRVHG

SEQ ID NO: 33 - protein, 6 aa, synthetic construct
  REGION 1..6: note = Clone 802 CDRL3
DYGFPL

SEQ ID NO: 34 - protein, 6 aa, synthetic construct
  REGION 1..6: note = Clone 905 CDRH1
SSYLMH

SEQ ID NO: 35 - protein, 10 aa, synthetic construct
  REGION 1..10: note = Clone 905 CDRH2
VISGSGGSTR

SEQ ID NO: 36 - protein, 8 aa, synthetic construct
  REGION 1..8: note = Clone 905 CDRH3
DLYRRVAG

SEQ ID NO: 37 - protein, 6 aa, synthetic construct
  REGION 1..6: note = Clone 905 CDRL3
DYALPL

SEQ ID NO: 38 - protein, 6 aa, synthetic construct
  REGION 1..6: note = Clone 906 CDRH1
SNYAMH

SEQ ID NO: 39 - protein, 10 aa, synthetic construct
  REGION 1..10: note = Clone 906 CDRH2
AISGNGGSTH

SEQ ID NO: 40 - protein, 8 aa, synthetic construct
  REGION 1..8: note = Clone 906 CDRH3
DRFRRVYG

SEQ ID NO: 41 - protein, 6 aa, synthetic construct
  REGION 1..6: note = Clone 906 CDRL3
DYTFPL

SEQ ID NO: 42 - protein, 6 aa, synthetic construct
  REGION 1..6: note = Clone 817 CDRH1
SSYAMH

SEQ ID NO: 43 - protein, 10 aa, synthetic construct
  REGION 1..10: note = Clone 817 CDRH2
AISGSGGSTR

SEQ ID NO: 44 - protein, 7 aa, synthetic construct
  REGION 1..7: note = Clone 817 CDRH3
GRWSKWG

SEQ ID NO: 45 - protein, 6 aa, synthetic construct
  REGION 1..6: note = Clone 817 CDRL3
TDNFPY

SEQ ID NO: 46 - protein, 8 aa, synthetic construct
DYKDDDDK

SEQ ID NO: 47 - protein, 10 aa, synthetic construct
EQKLISEEDL

SEQ ID NO: 48 - protein, 5 aa, synthetic construct
GGSGG

SEQ ID NO: 49 - protein, 9 aa, synthetic construct
FNFSSYVMH

SEQ ID NO: 50 - protein, 9 aa, synthetic construct
FSFSHYAMH

SEQ ID NO: 51 - protein, 9 aa, synthetic construct
FSLSDYYMN

SEQ ID NO: 52 - protein, 9 aa, synthetic construct
FTFNIFVMS

SEQ ID NO: 53 - protein, 9 aa, synthetic construct
FTFNDYAMH

SEQ ID NO: 54 - protein, 9 aa, synthetic construct
FTFSSYGMH

SEQ ID NO: 55 - protein, 9 aa, synthetic construct
FTFSSHDMH

SEQ ID NO: 56 - protein, 9 aa, synthetic construct
FTFSGYGMH

SEQ ID NO: 57 - protein, 9 aa, synthetic construct
FTFRHHGMT

SEQ ID NO: 58 - protein, 9 aa, synthetic construct
FTFSTFSMN

SEQ ID NO: 59 - protein, 9 aa, synthetic construct
FTFSSYAMH

SEQ ID NO: 60 - protein, 9 aa, synthetic construct
FTFRMYATH

SEQ ID NO: 61 - protein, 9 aa, synthetic construct
FTFRNYAMH

SEQ ID NO: 62 - protein, 9 aa, synthetic construct
FTFGSYAFH

SEQ ID NO: 63 - protein, 9 aa, synthetic construct
FTFZZYZMZ

SEQ ID NO: 64 - protein, 11 aa, synthetic construct
SAISSDGETTY

SEQ ID NO: 65 - protein, 11 aa, synthetic construct
AVISYDGENTY

SEQ ID NO: 66 - protein, 11 aa, synthetic construct
AYISSSSGYTN

SEQ ID NO: 67 - protein, 11 aa, synthetic construct
SGVFGSGGNTD

SEQ ID NO: 68 - protein, 11 aa, synthetic construct
SGISWDSSSIG

SEQ ID NO: 69 - protein, 11 aa, synthetic construct
AVMYYDGSNKD

SEQ ID NO: 70 - protein, 10 aa, synthetic construct
GIGTAGDTYY

SEQ ID NO: 71 - protein, 11 aa, synthetic construct
ALISYDESNKY

SEQ ID NO: 72 - protein, 11 aa, synthetic construct
ASLSGSGTKTH

SEQ ID NO: 73 - protein, 11 aa, synthetic construct
SYISRTSKTIY

SEQ ID NO: 74 - protein, 11 aa, synthetic construct
AVISSDGGNKY

SEQ ID NO: 75 - protein, 11 aa, synthetic construct
ALISYDGSNKY

SEQ ID NO: 76 - protein, 11 aa, synthetic construct
ALIKYDGRNKY

SEQ ID NO: 77 - protein, 11 aa, synthetic construct
AFISYNGSSKY

SEQ ID NO: 78 - protein, 11 aa, synthetic construct
AZIZZZGZZTZ

SEQ ID NO: 79 - protein, 9 aa, synthetic construct
RDRYNAFDV

SEQ ID NO: 80 - protein, 9 aa, synthetic construct
RDRIYGMDV

SEQ ID NO: 81 - protein, 9 aa, synthetic construct
RDRDGYYKH

SEQ ID NO: 82 - protein, 9 aa, synthetic construct
KHRVTGFDS

SEQ ID NO: 83 - protein, 9 aa, synthetic construct
KGRDVAFDI

SEQ ID NO: 84 - protein, 9 aa, synthetic construct
REKDYGLDV

SEQ ID NO: 85 - protein, 9 aa, synthetic construct
RDRYYGMDV

SEQ ID NO: 86 - protein, 9 aa, synthetic construct
KVKFAPNDY

SEQ ID NO: 87 - protein, 9 aa, synthetic construct
KAKRGYFDL

SEQ ID NO: 88 - protein, 7 aa, synthetic construct
RGRFFDY

SEQ ID NO: 89 - protein, 9 aa, synthetic construct
RGNPGGGDY

SEQ ID NO: 90 - protein, 9 aa, synthetic construct
RDLGGIMDV

SEQ ID NO: 91 - protein, 9 aa, synthetic construct
RDIGYGPDY

SEQ ID NO: 92 - protein, 9 aa, synthetic construct
RAPDGAFGY

SEQ ID NO: 93 - protein, 8 aa, synthetic construct
  VARIANT 4: note = X can be any amino acid
RZZXZFDV

SEQ ID NO: 94 - protein, 11 aa, synthetic construct
QQYDNLGDLSF

SEQ ID NO: 95 - protein, 11 aa, synthetic construct
QQYDNLPPLTF

SEQ ID NO: 96 - protein, 9 aa, synthetic construct
QQYDKLPTF

SEQ ID NO: 97 - protein, 10 aa, synthetic construct
QQYQNLPLTF

SEQ ID NO: 98 - protein, 8 aa, synthetic construct
QQYNSYSF

SEQ ID NO: 99 - protein, 10 aa, synthetic construct
LQHNSNPLTF

SEQ ID NO: 100 - protein, 9 aa, synthetic construct
KQYADYWTF

SEQ ID NO: 101 - protein, 10 aa, synthetic construct
QQSYSAPRTF

SEQ ID NO: 102 - protein, 10 aa, synthetic construct
QQYHSYPWTF

SEQ ID NO: 103 - protein, 10 aa, synthetic construct
QQSVMIPMTF

SEQ ID NO: 104 - protein, 8 aa, synthetic construct
QQNSNWTF

SEQ ID NO: 105 - protein, 10 aa, synthetic construct
QQANSFPLTF

SEQ ID NO: 106 - protein, 11 aa, synthetic construct
QQHQNVPLTTF

SEQ ID NO: 107 - protein, 10 aa, synthetic construct
QHYDDFPISF

SEQ ID NO: 108 - protein, 10 aa, synthetic construct
QQZZZZPZTF

SEQ ID NO: 109 - protein, 98 aa, synthetic construct
  VARIANT 5: note = X can be V or L
  VARIANT 10: note = X can be G or V
  VARIANT 11: note = X can be L or V
  VARIANT 13: note = X can be Q, K or R
  VARIANT 16: note = X can be G or R
  VARIANT 30..31: note = X can be S or D
  VARIANT 33: note = X can be A, G, N or W
  VARIANT 35: note = X can be H, S or N
  VARIANT 46: note = X can be E or V
  VARIANT 47: note = X can be W or Y
  VARIANT 49: note = X can be S or A
  VARIANT 50: note = X can be V, A,L or V
  VARIANT 52: note = X can be S, N, K, W or V
  VARIANT 53: note = X can be S, W, Y or G
  VARIANT 54: note = X can be D,S or N
  VARIANT 55: note = X can be G or S
  VARIANT 56: note = X can be S or G
  VARIANT 57: note = X can be S,N,T,D or V
  VARIANT 58: note = X can be T,K or I
  VARIANT 59: note = X can be Y, G or S
  VARIANT 61: note = X can be A or V
  VARIANT 75: note = X can be S or A
  VARIANT 78: note = X can be T or S
  VARIANT 84: note = X can be N or G
  VARIANT 88: note = X can be A or T
  VARIANT 91: note = X can be T or M
  VARIANT 95: note = X can be Y or H
  VARIANT 98: note = X can be R or K
ZVQLXESGGXXVXPGXSLRLSCAASGFTFXXYXMXWVRQAPGKGLXXVXXXXXXXXXXXYXBSVKGRFTISRDNXKNXLYLQMXSLRXEDXACYXCAX

SEQ ID NO: 110 - DNA, 36 bp, synthetic construct
  source 1..36: mol_type = other DNA
tcagctattagtggtagtggaggtagtacttactac

SEQ ID NO: 111 - DNA, 61 bp, synthetic construct
  source 1..61: mol_type = other DNA
ggcttaggtctctccgtgrtckcnnknnknnknnkgstttcgcgagacgaggtctgaacgg

SEQ ID NO: 112 - DNA, 64 bp, synthetic construct
  source 1..64: mol_type = other DNA
ggcttaggtctctccgtgrtckcnnknnknnknnknnkgstttcgcgagacgaggtctgaacgg

SEQ ID NO: 113 - DNA, 67 bp, synthetic construct
  source 1..67: mol_type = other DNA
ggcttaggtctctccgtgrtckcnnknnknnknnknnknnkgstttcgcgagacgaggtctgaacgg

SEQ ID NO: 114 - DNA, 70 bp, synthetic construct
  source 1..70: mol_type = other DNA
ggcttaggtctctccgtgrtckcnnknnknnknnknnknnknnkgstttcgcgagacgaggtctgaacgg

SEQ ID NO: 115 - DNA, 73 bp, synthetic construct
  source 1..73: mol_type = other DNA
ggcttaggtctctccgtgrtckcnnknnknnknnknnknnknnknnkgstttcgcgagacgaggtctgaacgg

SEQ ID NO: 116 - DNA, 76 bp, synthetic construct
  source 1..76: mol_type = other DNA
ggcttaggtctctccgtgrtckcnnknnknnknnknnknnknnknnknnkgstttcgcgagacgaggtctgaacgg

SEQ ID NO: 117 - DNA, 79 bp, synthetic construct
  source 1..79: mol_type = other DNA
ggcttaggtctctccgtgrtckcnnknnknnknnknnknnknnknnknnknnkgstttcgcgagacgaggtctgaacgg

SEQ ID NO: 118 - DNA, 33 bp, synthetic construct
  source 1..33: mol_type = other DNA
gaaagtccaaggaacancataccactgctggca

SEQ ID NO: 119 - protein, 9 aa, synthetic construct
  VARIANT 3: note = X can be Y,D,L,A,H,S,F,R,T,W or G
  VARIANT 4: note = X can be Y,N,D,S,T or A
  VARIANT 5: note = X can be S,N,T,A,D or G
  VARIANT 6: note = X can be Y,F,A,L,T,S,H,W,I,N,R,V,D or G
  VARIANT 8: note = X can be L,Y,W,F or R
QQXXXXPXT

SEQ ID NO: 120 - protein, 20 aa, synthetic construct
GGGGSGGGGSGGGGSGGGGS